European Patent Specification EP 3 628 684 B1, published September 18, 2024. Title: Determining Antigen Recognition through Barcoding of MHC Multimers. Applicant: Immudex ApS Herlev Hospital. The sequence listing filed with the application follows.

SEQUENCE LISTING (189 sequences)

SEQ ID NO: 1 - DNA, 69 bp, Artificial sequence
  Barcode for CMV, Biotin-TEG at 5' end
  misc_feature (1)..(69): Barcode for CMV
  misc_feature (13)..(18): n: any of A, T, G, C independently
gagatacgttgacctcgttgaannnnnntctatccattccatccagctcacttaagctcttggttgcat

SEQ ID NO: 2 - DNA, 69 bp, Artificial sequence
  Barcode for HIV, Biotin-TEG at 5' end
  misc_feature (1)..(69): Barcode for HIV
  misc_feature (13)..(18): n: any of A, T, G, C independently
gagatacgttgacctcgttgaannnnnntctataggtgtctactacctcacttaagctcttggttgcat

SEQ ID NO: 3 - DNA, 20 bp, Artificial sequence
  Forward-01 primer
  primer_bind (1)..(20): Forward-01 primer
gagatacgttgacctcgttg

SEQ ID NO: 4 - DNA, 20 bp, Artificial sequence
  Reverse-01 primer
  primer_bind (1)..(20): Reverse-01 primer
atgcaaccaagagcttaagt

SEQ ID NO: 5 - DNA, 69 bp, Artificial sequence; identical to SEQ ID NO: 1
  TestOligo-01, biotin-TEG at 5' end
  misc_feature (1)..(69): TestOligo-01
  misc_feature (13)..(18): n: any of A, T, G, C independently

SEQ ID NO: 6 - DNA, 69 bp, Artificial sequence; identical to SEQ ID NO: 1
  TestOligo-02, biotin-TEG at 5' end followed by HEG (terminal modifications)
  misc_feature (1)..(69): TestOligo-02
  misc_feature (13)..(18): n: any of A, T, G, C independently

SEQ ID NO: 7 - DNA, 69 bp, Artificial sequence; identical to SEQ ID NO: 1
  TestOligo-03, biotin-TEG at 5' end followed by HEG (terminal modifications) and HEG at 3' end
  misc_feature (1)..(69): TestOligo-03
  misc_feature (13)..(18): n: any of A, T, G, C independently

SEQ ID NO: 8 - DNA, 69 bp, Artificial sequence
  TestOligo-04, biotin-TEG at 5' end followed by HEG (terminal modifications) and HEG at 3' end
  misc_feature (1)..(69): TestOligo-04
  misc_feature (13)..(18): n: any of A, T, G, C independently
gagatacgttgacctcgttgaannnnnntcttgaactatgaatcgtctcacttaagctcttggttgcat

SEQ ID NO: 9 - DNA, 69 bp, Artificial sequence; identical to SEQ ID NO: 2
  TestOligo-05, biotin-TEG at 5' end followed by HEG (terminal modifications) and HEG at 3' end
  misc_feature (1)..(69): TestOligo-05
  misc_feature (13)..(18): n: any of A, T, G, C

SEQ ID NO: 10 - DNA, 69 bp, Artificial sequence
  TestOligo-06, biotin-TEG at 5' end followed by HEG (terminal modifications) and HEG at 3' end
  misc_feature (1)..(69): TestOligo-06
  misc_feature (13)..(18): n: any of A, T, G, C independently
gagatacgttgacctcgttgaannnnnntctttattggagagcacgctcacttaagctcttggttgcat

SEQ ID NO: 11 - DNA, 19 bp, Artificial sequence
  LNA-3, 6FAM in 5', BHQ-1-plus in 3'
  misc_feature (1)..(19): LNA-3
  misc_feature (4)..(6): LNA modified RNA nucleotides
  misc_feature (9)..(10): LNA modified RNA nucleotides
  misc_feature (13)..(15): LNA modified RNA nucleotides
tctatccattccatccagc

SEQ ID NO: 12 - DNA, 19 bp, Artificial sequence
  LNA-4, 6FAM in 5'. BHQ-1-plus in 3'
  misc_feature (1)..(19): LNA-4
  misc_feature (4)..(6): LNA modified RNA nucleotides
  misc_feature (9)..(10): LNA modified RNA nucleotides
  misc_feature (13)..(15): LNA modified RNA nucleotides
tcttgaactatgaatcgtc

SEQ ID NO: 13 - DNA, 19 bp, Artificial sequence
  LNA-5, HEX in 5', BHQ-1-plus in 3'
  misc_feature (1)..(19): LNA-5
  misc_feature (4)..(6): LNA modified RNA nucleotides
  misc_feature (9)..(10): LNA modified RNA nucleotides
  misc_feature (13)..(15): LNA modified RNA nucleotides
tctataggtgtctactacc

SEQ ID NO: 14 - DNA, 19 bp, Artificial sequence
  LNA-6, cyanine 5 in 5'-end; bhq-2-plus in 3' end
  misc_feature (1)..(19): LNA-6
  misc_feature (4)..(6): LNA modified RNA nucleotides
  misc_feature (9)..(10): LNA modified RNA nucleotides
  misc_feature (13)..(15): LNA modified RNA nucleotides
tctttattggagagcacgc

SEQ ID NO: 15 - protein, 9 aa, Influenza virus
  PEPTIDE (1)..(9): Dextramer 1, Flu (HLA-A*0201/GILGFVFTL/MP/Influenza)
GILGFVFTL

SEQ ID NO: 16 - protein, 9 aa, Human cytomegalovirus
  PEPTIDE (1)..(9): Dextramer 2, CMV (HLA-A*0201/NLVPMVATV/pp65/CMV)
NLVPMVATV

SEQ ID NO: 17 - protein, 9 aa, Artificial sequence
  Negative control
  PEPTIDE (1)..(9): Dextramer 3, Negative (HLA-A*0201/ALIAPVHAV/Neg.Control).
ALIAPVHAV

SEQ ID NO: 18 - protein, 9 aa, Human immunodeficiency virus
  PEPTIDE (1)..(9): HIV derived peptide
ILKEPVHGV

SEQ ID NO: 19 - protein, 10 aa, Human cytomegalovirus
  PEPTIDE (1)..(10): CMV-derived peptide
TPRVTGGGAM

SEQ ID NO: 20 - DNA, 20 bp, Artificial sequence
  Reverse-03, HEG at 5'
  misc_feature (1)..(20): Reverse-03
atgcaaccaagagcttaagt

SEQ ID NO: 21 - DNA, 21 bp, Artificial sequence
  Probe-03 FAM at 5'. BHQ-1-plus at 3'
  misc_feature (1)..(21): Probe-03 FAM at 5'
tctatccattccatccagctc

SEQ ID NO: 22 - DNA, 21 bp, Artificial sequence
  Probe-04 FAM at 5'. BHQ-1-plus at 3'
  misc_feature (1)..(21): Probe-04
tcttgaactatgaatcgtctc

SEQ ID NO: 23 - DNA, 21 bp, Artificial sequence
  Probe-05 HEX at 5'. BHQ-1-plus at 3'
  misc_feature (1)..(21): Probe-05 HEX at 5'
tctataggtgtctactacctc

SEQ ID NO: 24 - DNA, 21 bp, Artificial sequence
  Probe-06 cyanine 5 in 5'-end; bhq-2-plus in 3' end
  misc_feature (1)..(21): Probe-06
tctttattggagagcacgctc

SEQ ID NO: 25 - DNA, 58 bp, Artificial sequence
  A-key 1OS-F1-1
  misc_feature (1)..(58): A-key 1OS-F1-1
ccatctcatccctgcgtgtctccgactcaggaagatgattctataaactgtgcggtcc

SEQ ID NO: 26 - DNA, 58 bp, Artificial sequence
  A-key 1OS-F1-2
  misc_feature (1)..(58): A-key 1OS-F1-2
ccatctcatccctgcgtgtctccgactcagtcctgagattctataaactgtgcggtcc

SEQ ID NO: 27 - DNA, 58 bp, Artificial sequence
  A-key 1OS-F1-3
  misc_feature (1)..(58): A-key 1OS-F1-3
ccatctcatccctgcgtgtctccgactcagtgtggagattctataaactgtgcggtcc

SEQ ID NO: 28 - DNA, 58 bp, Artificial sequence
  A-key 1OS-F1-4
  misc_feature (1)..(58): A-key 1OS-F1-4
ccatctcatccctgcgtgtctccgactcagcatttagattctataaactgtgcggtcc

SEQ ID NO: 29 - DNA, 58 bp, Artificial sequence
  A-key 1OS-F1-5
  misc_feature (1)..(58): A-key 1OS-F1-5
ccatctcatccctgcgtgtctccgactcagttacccgattctataaactgtgcggtcc

SEQ ID NO: 30 - DNA, 58 bp, Artificial sequence
  A-key 1OS-F1-6
  misc_feature (1)..(58): A-key 1OS-F1-6
ccatctcatccctgcgtgtctccgactcagattctcgattctataaactgtgcggtcc

SEQ ID NO: 31 - DNA, 58 bp, Artificial sequence
  A-key 1OS-F1-7
  misc_feature (1)..(58): A-key 1OS-F1-7
ccatctcatccctgcgtgtctccgactcagagacccgattctataaactgtgcggtcc

SEQ ID NO: 32 - DNA, 58 bp, Artificial sequence
  A-key 1OS-F1-8
  misc_feature (1)..(58): A-key 1OS-F1-8
ccatctcatccctgcgtgtctccgactcagcgcatggattctataaactgtgcggtcc

SEQ ID NO: 33 - DNA, 58 bp, Artificial sequence
  A-key 1OS-F1-9
  misc_feature (1)..(58): A-key 1OS-F1-9
ccatctcatccctgcgtgtctccgactcagtcctcggattctataaactgtgcggtcc

SEQ ID NO: 34 - DNA, 58 bp, Artificial sequence
  A-key 1OS-F1-10
  misc_feature (1)..(58): A-key 1OS-F1-10
ccatctcatccctgcgtgtctccgactcagattcctgattctataaactgtgcggtcc

SEQ ID NO: 35 - DNA, 58 bp, Artificial sequence
  A-key 1OS-F1-11
  misc_feature (1)..(58): A-key 1OS-F1-11
ccatctcatccctgcgtgtctccgactcagcgtcgagattctataaactgtgcggtcc

SEQ ID NO: 36 - DNA, 58 bp, Artificial sequence
  A-key 1OS-F1-12
  misc_feature (1)..(58): A-key 1OS-F1-12
ccatctcatccctgcgtgtctccgactcaggccaatgattctataaactgtgcggtcc

SEQ ID NO: 37 - DNA, 58 bp, Artificial sequence
  A-key 1OS-F1-13
  misc_feature (1)..(58): A-key 1OS-F1-13
ccatctcatccctgcgtgtctccgactcagatacgggattctataaactgtgcggtcc

SEQ ID NO: 38 - DNA, 58 bp, Artificial sequence
  A-key 1OS-F1-14
  misc_feature (1)..(58): A-key 1OS-F1-14
ccatctcatccctgcgtgtctccgactcaggtcagagattctataaactgtgcggtcc

SEQ ID NO: 39 - DNA, 58 bp, Artificial sequence
  A-key 1OS-F1-15
  misc_feature (1)..(58): A-key 1OS-F1-15
ccatctcatccctgcgtgtctccgactcagcgagttgattctataaactgtgcggtcc

SEQ ID NO: 40 - DNA, 54 bp, Artificial sequence
  A-key 2OS-F1-1
  misc_feature (1)..(54): A-key 2OS-F1-1
ccatctcatccctgcgtgtctccgactcagctgggggaagttccagccagcgtc

SEQ ID NO: 41 - DNA, 54 bp, Artificial sequence
  A-key 2OS-F1-2
  misc_feature (1)..(54): A-key 2OS-F1-2
ccatctcatccctgcgtgtctccgactcagctccacgaagttccagccagcgtc

SEQ ID NO: 42 - DNA, 54 bp, Artificial sequence
  A-key 2OS-F1-3
  misc_feature (1)..(54): A-key 2OS-F1-3
ccatctcatccctgcgtgtctccgactcagcttaccgaagttccagccagcgtc

SEQ ID NO: 43 - DNA, 54 bp, Artificial sequence
  A-key 2OS-F1-4
  misc_feature (1)..(54): A-key 2OS-F1-4
ccatctcatccctgcgtgtctccgactcagtggcaggaagttccagccagcgtc

SEQ ID NO: 44 - DNA, 54 bp, Artificial sequence
  A-key 2OS-F1-5
  misc_feature (1)..(54): A-key 2OS-F1-5
ccatctcatccctgcgtgtctccgactcagtgagtagaagttccagccagcgtc

SEQ ID NO: 45 - DNA, 54 bp, Artificial sequence
  A-key 2OS-F1-6
  misc_feature (1)..(54): A-key 2OS-F1-6
ccatctcatccctgcgtgtctccgactcagattcaggaagttccagccagcgtc

SEQ ID NO: 46 - DNA, 54 bp, Artificial sequence
  A-key 2OS-F1-7
  misc_feature (1)..(54): A-key 2OS-F1-7
ccatctcatccctgcgtgtctccgactcagtgagctgaagttccagccagcgtc

SEQ ID NO: 47 - DNA, 54 bp, Artificial sequence
  A-key 2OS-F1-8
  misc_feature (1)..(54): A-key 2OS-F1-8
ccatctcatccctgcgtgtctccgactcagggcgtggaagttccagccagcgtc

SEQ ID NO: 48 - DNA, 54 bp, Artificial sequence
  A-key 2OS-F1-9
  misc_feature (1)..(54): A-key 2OS-F1-9
ccatctcatccctgcgtgtctccgactcagaaattggaagttccagccagcgtc

SEQ ID NO: 49 - DNA, 54 bp, Artificial sequence
  A-key 2OS-F1-10
  misc_feature (1)..(54): A-key 2OS-F1-10
ccatctcatccctgcgtgtctccgactcaggctgacgaagttccagccagcgtc

SEQ ID NO: 50 - DNA, 54 bp, Artificial sequence
  A-key 2OS-F1-11
  misc_feature (1)..(54): A-key 2OS-F1-11
ccatctcatccctgcgtgtctccgactcagttcttagaagttccagccagcgtc

SEQ ID NO: 51 - DNA, 54 bp, Artificial sequence
  A-key 2OS-F1-12
  misc_feature (1)..(54): A-key 2OS-F1-12
ccatctcatccctgcgtgtctccgactcagtggtgggaagttccagccagcgtc

SEQ ID NO: 52 - DNA, 54 bp, Artificial sequence
  A-key 2OS-F1-13
  misc_feature (1)..(54): A-key 2OS-F1-13
ccatctcatccctgcgtgtctccgactcaggcagtcgaagttccagccagcgtc

SEQ ID NO: 53 - DNA, 54 bp, Artificial sequence
  A-key 2OS-F1-14
  misc_feature (1)..(54): A-key 2OS-F1-14
ccatctcatccctgcgtgtctccgactcagtcgtgagaagttccagccagcgtc

SEQ ID NO: 54 - DNA, 54 bp, Artificial sequence
  A-key 2OS-F1-15
  misc_feature (1)..(54): A-key 2OS-F1-15
ccatctcatccctgcgtgtctccgactcagtacagtgaagttccagccagcgtc

SEQ ID NO: 55 - DNA, 44 bp, Artificial sequence
  P1-key 1OS-R1
  misc_feature (1)..(44): P1-key 1OS-R1
cctctctatgggcagtcggtgatgagtacatgatagcgccgtac

SEQ ID NO: 56 - DNA, 44 bp, Artificial sequence
  P1-key 2OS-R1
  misc_feature (1)..(44): P1-key 2OS-R1
cctctctatgggcagtcggtgatctgtgactatgtgaggctttc

SEQ ID NO: 57 - DNA, 81 bp, Artificial sequence
  1OS-1-Oligo-1, Biotin-C6- in 5'
  misc_feature (1)..(81): 1OS-1-Oligo-1
  misc_feature (26)..(31): n: any of A, T, G, C independently
agattctataaactgtgcggtccttnnnnnntatgaggacgaatctcccgcttataggtacggcgctatcatgtactcatg

SEQ ID NO: 58 - DNA, 81 bp, Artificial sequence
  1OS-1-Oligo-2, Biotin-C6- in 5'
  misc_feature (1)..(81): 1OS-1-Oligo-2, Biotin-C6- in 5'
  misc_feature (26)..(31): n: any of A, T, G, C independently
agattctataaactgtgcggtccttnnnnnnggtcttgacaaacgtgtgcttgtacggtacggcgctatcatgtactcatg

SEQ ID NO: 59 - DNA, 81 bp, Artificial sequence
  1OS-1-Oligo-3, Biotin-C6- in 5'
  misc_feature (1)..(81): 1OS-1-Oligo-3
  misc_feature (26)..(31): n: any of A, T, G, C independently
agattctataaactgtgcggtccttnnnnnngtttatcgggcgtggtgctcgcataggtacggcgctatcatgtactcatg

SEQ ID NO: 60 - DNA, 81 bp, Artificial sequence
  1OS-1-Oligo-4, Biotin-C6- in 5'
  misc_feature (1)..(81): 1OS-1-Oligo-4, Biotin-C6- in 5'
  misc_feature (26)..(31): n: any of A, T, G, C independently
agattctataaactgtgcggtccttnnnnnnccgatgttgacggactaatcctgacggtacggcgctatcatgtactcatg

SEQ ID NO: 61 - DNA, 81 bp, Artificial sequence
  1OS-1-Oligo-5, Biotin-C6- in 5'
  misc_feature (1)..(81): 1OS-1-Oligo-5, Biotin-C6- in 5'
  misc_feature (26)..(31): n: any of A, T, G, C independently
agattctataaactgtgcggtccttnnnnnntagtagttcagacgccgttaagcgcggtacggcgctatcatgtactcatg

SEQ ID NO: 62 - DNA, 81 bp, Artificial sequence
  1OS-1-Oligo-6, Biotin-C6- in 5'
  misc_feature (1)..(81): 1OS-1-Oligo-4
  misc_feature (26)..(31): n: any of A, T, G, C independently
agattctataaactgtgcggtccttnnnnnnccgtacctagatacactcaatttgtggtacggcgctatcatgtactcatg

SEQ ID NO: 63 - DNA, 81 bp, Artificial sequence
  1OS-1-Oligo-7, Biotin-C6- in 5'
  misc_feature (1)..(81): 1OS-1-Oligo-7
  misc_feature (26)..(31): n: any of A, T, G, C independently
agattctataaactgtgcggtccttnnnnnnggggttccgttttacattccaggaaggtacggcgctatcatgtactcatg

SEQ ID NO: 64 - DNA, 81 bp, Artificial sequence
  1OS-1-Oligo-8, Biotin-C6- in 5'
  misc_feature (1)..(81): 1OS-1-Oligo-8
  misc_feature (26)..(31): n: any of A, T, G, C independently
agattctataaactgtgcggtccttnnnnnntatcccgtgaagcttgagtggaatcggtacggcgctatcatgtactcatg

SEQ ID NO: 65 - DNA, 81 bp, Artificial sequence
  1OS-1-Oligo-9, Biotin-C6- in 5'
  misc_feature (1)..(81): 1OS-1-Oligo-9
  misc_feature (26)..(31): n: any of A, T, G, C independently
agattctataaactgtgcggtccttnnnnnnctgacgtgtgaggcgctagagcataggtacggcgctatcatgtactcatg

SEQ ID NO: 66 - DNA, 81 bp, Artificial sequence
  1OS-1-Oligo-10, Biotin-C6- in 5'
  misc_feature (1)..(81): 1OS-1-Oligo-10
  misc_feature (26)..(31): n: any of A, T, G, C independently
agattctataaactgtgcggtccttnnnnnnggtatggcacgcctaatctggacacggtacggcgctatcatgtactcatg

SEQ ID NO: 67 - DNA, 72 bp, Artificial sequence
  2OS-1-Oligo-A1, Biotin-C6- in 5'
  misc_feature (1)..(72): 2OS-1-Oligo-A1
  misc_feature (26)..(31): n: any of A, T, G, C independently
gaagttccagccagcgtcacagtttnnnnnncgagggcaatggttaactgacacgtggtcagcatcatttcc

SEQ ID NO: 68 - DNA, 72 bp, Artificial sequence
  2OS-1-Oligo-A2, Biotin-C6- in 5'
  misc_feature (1)..(72): 2OS-1-Oligo-A2
  misc_feature (26)..(31): n: any of A, T, G, C independently
gaagttccagccagcgtcacagtttnnnnnncagaaagcagtctcgtcggttcgaaggtcagcatcatttcc

SEQ ID NO: 69 - DNA, 72 bp, Artificial sequence
  2OS-1-Oligo-A3, Biotin-C6- in 5'
  misc_feature (1)..(72): 2OS-1-Oligo-A3
  misc_feature (26)..(31): n: any of A, T, G, C indepepndently
gaagttccagccagcgtcacagtttnnnnnntaagtagcgggcataatgtacgctcggtcagcatcatttcc

SEQ ID NO: 70 - DNA, 72 bp, Artificial sequence
  2OS-1-Oligo-A4, Biotin-C6- in 5'
  misc_feature (1)..(72): 2OS-1-Oligo-A4
  misc_feature (26)..(31): n: any of A, T, G, C independently
gaagttccagccagcgtcacagtttnnnnnnggatccagtaagctactgcgtttatggtcagcatcatttcc

SEQ ID NO: 71 - DNA, 72 bp, Artificial sequence
  2OS-1-Oligo-A5, Biotin-C6- in 5'
  misc_feature (1)..(72): 2OS-1-Oligo-A5
  misc_feature (26)..(31): n: any of A, T, G, C independently
gaagttccagccagcgtcacagtttnnnnnngggctgcggagcgtttactctgtatggtcagcatcatttcc

SEQ ID NO: 72 - DNA, 72 bp, Artificial sequence
  2OS-1-Oligo-A6
  misc_feature (1)..(72): 2OS-1-Oligo-A6
  misc_feature (26)..(31): n: any of A, T, G, C independently
gaagttccagccagcgtcacagtttnnnnnnaaacgtatgtgctttgtcggatgccggtcagcatcatttcc

SEQ ID NO: 73 - DNA, 72 bp, Artificial sequence
  2OS-1-Oligo-B1
  misc_feature (1)..(72): 2OS-1-Oligo-B1
  misc_feature (26)..(31): n: any of A, T, G, C independently
ctgtgactatgtgaggctttctcgannnnnngcctgtagtcccacgcgatctaacaggaaatgatgctgacc

SEQ ID NO: 74 - DNA, 72 bp, Artificial sequence
  2OS-1-Oligo-B2
  misc_feature (1)..(72): 2OS-1-Oligo-B2
  misc_feature (26)..(31): n: any of A, T, G, C
ctgtgactatgtgaggctttctcgannnnnncaaccattgattggggacaactgggggaaatgatgctgacc

SEQ ID NO: 75 - DNA, 72 bp, Artificial sequence
  2OS-1-Oligo-B3
  misc_feature (1)..(72): 2OS-1-Oligo-B2
  misc_feature (26)..(31): n: any of A, T, G, C independently
ctgtgactatgtgaggctttctcgannnnnnacgtttaagcatctgtactccagatggaaatgatgctgacc

SEQ ID NO: 76 - DNA, 72 bp, Artificial sequence
  2OS-1-Oligo-B4
  misc_feature (1)..(72): 2OS-1-Oligo-B4
  misc_feature (26)..(31): n: any of A, T, G, C independently
ctgtgactatgtgaggctttctcgannnnnngaattgaagccatcgtttcgcgcaaggaaatgatgctgacc

SEQ ID NO: 77 - DNA, 72 bp, Artificial sequence
  2OS-1-Oligo-B5
  misc_feature (1)..(72): 2OS-1-Oligo-B5
  misc_feature (26)..(31): n: any of A, T, G, C independently
ctgtgactatgtgaggctttctcgannnnnncgtagcttttgtagcgtctgagggcggaaatgatgctgacc

SEQ ID NO: 78 - DNA, 72 bp, Artificial sequence
  2OS-1-Oligo-B6
  misc_feature (1)..(72): 2OS-1-Oligo-B6
  misc_feature (26)..(31): n: any of A, T, G, C independently
ctgtgactatgtgaggctttctcgannnnnnaatcgtcagtccctgtttcgacatcggaaatgatgctgacc

SEQ ID NO: 79 - DNA, 72 bp, Artificial sequence
  2OS-1-Oligo-B7
  misc_feature (1)..(72): 2OS-1-Oligo-B7
  misc_feature (26)..(31): n: any of A, T, G, C independently
ctgtgactatgtgaggctttctcgannnnnncggtggtaggtgatacttctgtaccggaaatgatgctgacc

SEQ ID NO: 80 - DNA, 72 bp, Artificial sequence
  2OS-1-Oligo-B8
  misc_feature (1)..(72): 2OS-1-Oligo-B8
  misc_feature (26)..(31): n: any of A, T, G, C independently
ctgtgactatgtgaggctttctcgannnnnntgactatcggggcgtgacatgagctggaaatgatgctgacc

SEQ ID NO: 81 - DNA, 72 bp, Artificial sequence
  2OS-1-Oligo-B9
  misc_feature (1)..(72): 2OS-1-Oligo-B9
  misc_feature (26)..(31): n: any of A, T, G, C independently
ctgtgactatgtgaggctttctcgannnnnngttggtgaaactaccgacgctttacggaaatgatgctgacc

SEQ ID NO: 82 - DNA, 72 bp, Artificial sequence
  2OS-1-Oligo-B10
  misc_feature (1)..(72): 2OS-1-Oligo-B10
  misc_feature (26)..(31): n: any of A, T, G, C independently
ctgtgactatgtgaggctttctcgannnnnnaatggaggtgcaggaatactctcgtggaaatgatgctgacc

SEQ ID NO: 83 - protein, 11 aa, Human cytomegalovirus
  PEPTIDE (1)..(11): CMV  pp65  YSE
YSEHPTFTSQY

SEQ ID NO: 84 - protein, 9 aa, Human cytomegalovirus
  PEPTIDE (1)..(9): CMV  pp50  VTE
VTEHDTLLY

SEQ ID NO: 85 - protein, 9 aa, Influenza virus
  PEPTIDE (1)..(9): FLU  BP-VSD
VSDGGPNLY

SEQ ID NO: 86 - protein, 10 aa, Human herpesvirus 4
  PEPTIDE (1)..(10): EBV-EBNA4
AVFDRKSDAK

SEQ ID NO: 87 - protein, 9 aa, Human cytomegalovirus
  PEPTIDE (1)..(9): HCMV pp65
GPISGHVLK

SEQ ID NO: 88 - protein, 9 aa, Merkel Cell Polyoma Virus
  PEPTIDE (1)..(9): VP1
DLQGLVLDY

SEQ ID NO: 89 - protein, 9 aa, Merkel Cell Polyoma Virus
  PEPTIDE (1)..(9): VP1
VLGRKMTPK

SEQ ID NO: 90 - protein, 9 aa, Merkel Cell Polyoma Virus
  PEPTIDE (1)..(9): VP1
VTLRKRWVK

SEQ ID NO: 91 - protein, 9 aa, Merkel Cell Polyoma Virus
  PEPTIDE (1)..(9): VP1
LVLDYQTEY

SEQ ID NO: 92 - protein, 9 aa, Merkel Cell Polyoma Virus
  PEPTIDE (1)..(9): VP1
GQEKTVYPK

SEQ ID NO: 93 - protein, 10 aa, Merkel Cell Polyoma Virus
  PEPTIDE (1)..(10): VP1
VTFQSNQQDK

SEQ ID NO: 94 - protein, 10 aa, Merkel Cell Polyoma Virus
  PEPTIDE (1)..(10): VP1
LKGPQKASQK

SEQ ID NO: 95 - protein, 11 aa, Merkel Cell Polyoma Virus
  PEPTIDE (1)..(11): VP1
NVASVPKLLVK

SEQ ID NO: 96 - protein, 9 aa, Merkel Cell Polyoma Virus
  PEPTIDE (1)..(9): VP1
TSNWYTYTY

SEQ ID NO: 97 - protein, 11 aa, Merkel Cell Polyoma Virus
  PEPTIDE (1)..(11): VP1
LVLDYQTEYPK

SEQ ID NO: 98 - protein, 11 aa, Merkel Cell Polyoma Virus
  PEPTIDE (1)..(11): VP1
TLRKRWVKNPY

SEQ ID NO: 99 - protein, 11 aa, Merkel Cell Polyoma Virus
  PEPTIDE (1)..(11): VP1
AVTFQSNQQDK

SEQ ID NO: 100 - protein, 11 aa, Merkel Cell Polyoma Virus
  PEPTIDE (1)..(11): VP1
PLKGPQKASQK

SEQ ID NO: 101 - protein, 9 aa, Merkel Cell Polyoma Virus
  PEPTIDE (1)..(9): VP1
RIYEGSEQL

SEQ ID NO: 102 - protein, 9 aa, Merkel Cell Polyoma Virus
  PEPTIDE (1)..(9): VP1
SLFSNLMPK

SEQ ID NO: 103 - protein, 10 aa, Merkel Cell Polyoma Virus
  PEPTIDE (1)..(10): VP1
KLLVKGGVEV

SEQ ID NO: 104 - protein, 11 aa, Merkel Cell Polyoma Virus
  PEPTIDE (1)..(11): VP1
SLINVHYWDMK

SEQ ID NO: 105 - protein, 10 aa, Merkel Cell Polyoma Virus
  PEPTIDE (1)..(10): HPV  E6 29-38
TIHDIILECV

SEQ ID NO: 106 - protein, 9 aa, Influenza virus
  PEPTIDE (1)..(9): FLU  MP 58-66 GIL
GILGFVFTL

SEQ ID NO: 107 - protein, 9 aa, Human herpesvirus 4
  PEPTIDE (1)..(9): EBV  LMP2  CLG
CLGGLLTMV

SEQ ID NO: 108 - protein, 9 aa, Human herpesvirus 4
  PEPTIDE (1)..(9): EBV  BMF1  GLC
GLCTLVAML

SEQ ID NO: 109 - protein, 9 aa, Human herpesvirus 4
  PEPTIDE (1)..(9): EBV  LMP2  FLY
FLYALALLL

SEQ ID NO: 110 - protein, 9 aa, Human herpesvirus 4
  PEPTIDE (1)..(9): EBV  BRLF1  YVL
YVLDHLIVV

SEQ ID NO: 111 - protein, 10 aa, Human papillomavirus
  PEPTIDE (1)..(10): HPV  E7 11-20
YMLDLQPETT

SEQ ID NO: 112 - protein, 9 aa, Human cytomegalovirus
  PEPTIDE (1)..(9): CMV  IE1  VLE
VLEETSVML

SEQ ID NO: 113 - protein, 9 aa, Merkel Cell Polyoma Virus
  PEPTIDE (1)..(9): VP1
GCCPNVASV

SEQ ID NO: 114 - protein, 9 aa, Merkel Cell Polyoma Virus
  PEPTIDE (1)..(9): VP1
SITQIELYL

SEQ ID NO: 115 - protein, 9 aa, Merkel Cell Polyoma Virus
  PEPTIDE (1)..(9): VP1
LQMWEAISV

SEQ ID NO: 116 - protein, 9 aa, Merkel Cell Polyoma Virus
  PEPTIDE (1)..(9): VP1
AISVKTEVV

SEQ ID NO: 117 - protein, 9 aa, Merkel Cell Polyoma Virus
  PEPTIDE (1)..(9): VP1
KMTPKNQGL

SEQ ID NO: 118 - protein, 9 aa, Merkel Cell Polyoma Virus
  PEPTIDE (1)..(9): VP1
TVLQFSNTL

SEQ ID NO: 119 - protein, 9 aa, Merkel Cell Polyoma Virus
  PEPTIDE (1)..(9): VP1
GLFISCADI

SEQ ID NO: 120 - protein, 10 aa, Merkel Cell Polyoma Virus
  PEPTIDE (1)..(10): VP1
LLVKGGVEVL

SEQ ID NO: 121 - protein, 10 aa, Merkel Cell Polyoma Virus
  PEPTIDE (1)..(10): VP1
ELYLNPRMGV

SEQ ID NO: 122 - protein, 10 aa, Merkel Cell Polyoma Virus
  PEPTIDE (1)..(10): VP1
NLPAYSVARV

SEQ ID NO: 123 - protein, 10 aa, Merkel Cell Polyoma Virus
  PEPTIDE (1)..(10): VP1
TLQMWEAISV

SEQ ID NO: 124 - protein, 10 aa, Merkel Cell Polyoma Virus
  PEPTIDE (1)..(10): VP1
QMWEAISVKT

SEQ ID NO: 125 - protein, 10 aa, Merkel Cell Polyoma Virus
  PEPTIDE (1)..(10): VP1
VVGISSLINV

SEQ ID NO: 126 - protein, 10 aa, Merkel Cell Polyoma Virus
  PEPTIDE (1)..(10): VP1
SLINVHYWDM

SEQ ID NO: 127 - protein, 10 aa, Merkel Cell Polyoma Virus
  PEPTIDE (1)..(10): VP1
HMFAIGGEPL

SEQ ID NO: 128 - protein, 10 aa, Merkel Cell Polyoma Virus
  PEPTIDE (1)..(10): VP1
FAIGGEPLDL

SEQ ID NO: 129 - protein, 10 aa, Merkel Cell Polyoma Virus
  PEPTIDE (1)..(10): VP1
NLINSLFSNL

SEQ ID NO: 130 - protein, 11 aa, Merkel Cell Polyoma Virus
  PEPTIDE (1)..(11): VP1
FLFKTSGKMAL

SEQ ID NO: 131 - protein, 11 aa, Merkel Cell Polyoma Virus
  PEPTIDE (1)..(11): VP1
ALHGLPRYFNV

SEQ ID NO: 132 - protein, 11 aa, Merkel Cell Polyoma Virus
  PEPTIDE (1)..(11): VP1
NLINSLFSNLM

SEQ ID NO: 133 - protein, 11 aa, Merkel Cell Polyoma Virus
  PEPTIDE (1)..(11): VP1
FLDKFGQEKTV

SEQ ID NO: 134 - protein, 10 aa, Merkel Cell Polyoma Virus
  PEPTIDE (1)..(10): VP1
VKGGVEVLSV

SEQ ID NO: 135 - protein, 10 aa, Human cytomegalovirus
  PEPTIDE (1)..(10): HCMV 248-256
AYAQKIFKIL

SEQ ID NO: 136 - protein, 9 aa, Human herpesvirus 4
  PEPTIDE (1)..(9): EBV LMP2
IYVLVMLVL

SEQ ID NO: 137 - protein, 9 aa, Human herpesvirus 4
  PEPTIDE (1)..(9): EBV BRLF1
TYPVLEEMF

SEQ ID NO: 138 - protein, 9 aa, Human herpesvirus 4
  PEPTIDE (1)..(9): EBV BMLF1
DYNFVKQLF

SEQ ID NO: 139 - protein, 11 aa, Human cytomegalovirus
  PEPTIDE (1)..(11): CMV  pp150  TTV
TTVYPPSSTAK

SEQ ID NO: 140 - protein, 8 aa, Influenza virus
  PEPTIDE (1)..(8): FLU  NP 265-273  ILR
ILRGSVAH

SEQ ID NO: 141 - protein, 9 aa, Human herpesvirus 4
  PEPTIDE (1)..(9): EBV  EBNA  3a  RLR
RLRAEAQVK

SEQ ID NO: 142 - protein, 10 aa, Human cytomegalovirus
  PEPTIDE (1)..(10): CMV  pp150  TVY
TVYPPSSTAK

SEQ ID NO: 143 - protein, 9 aa, Human herpesvirus 4
  PEPTIDE (1)..(9): EBV  BRLF1 148-56  RVR
RVRAYTYSK

SEQ ID NO: 144 - protein, 9 aa, Merkel Cell Polyoma Virus
  PEPTIDE (1)..(9): VP1
ASVPKLLVK

SEQ ID NO: 145 - protein, 10 aa, Merkel Cell Polyoma Virus
  PEPTIDE (1)..(10): VP1
CCPNVASVPK

SEQ ID NO: 146 - protein, 9 aa, Merkel Cell Polyoma Virus
  PEPTIDE (1)..(9): VP1
ITIETVLGR

SEQ ID NO: 147 - protein, 9 aa, Merkel Cell Polyoma Virus
  PEPTIDE (1)..(9): VP1
NTLTTVLLD

SEQ ID NO: 148 - protein, 9 aa, Merkel Cell Polyoma Virus
  PEPTIDE (1)..(9): VP1
ALHGLPRYF

SEQ ID NO: 149 - protein, 10 aa, Merkel Cell Polyoma Virus
  PEPTIDE (1)..(10): VP1
VASVPKLLVK

SEQ ID NO: 150 - protein, 9 aa, Merkel Cell Polyoma Virus
  PEPTIDE (1)..(9): VP1
VSGQPMEGK

SEQ ID NO: 151 - protein, 10 aa, Merkel Cell Polyoma Virus
  PEPTIDE (1)..(10): VP1
KASSTCKTPK

SEQ ID NO: 152 - protein, 10 aa, Merkel Cell Polyoma Virus
  PEPTIDE (1)..(10): VP1
KTPKRQCIPK

SEQ ID NO: 153 - protein, 10 aa, Merkel Cell Polyoma Virus
  PEPTIDE (1)..(10): VP1
YTYTYDLQPK

SEQ ID NO: 154 - protein, 10 aa, Merkel Cell Polyoma Virus
  PEPTIDE (1)..(10): VP1
PITIETVLGR

SEQ ID NO: 155 - protein, 9 aa, Merkel Cell Polyoma Virus
  PEPTIDE (1)..(9): VP1
SVARVSLPM

SEQ ID NO: 156 - protein, 10 aa, Merkel Cell Polyoma Virus
  PEPTIDE (1)..(10): VP1
NSLFSNLMPK

SEQ ID NO: 157 - protein, 10 aa, Merkel Cell Polyoma Virus
  PEPTIDE (1)..(10): VP1
KVSGQPMEGK

SEQ ID NO: 158 - protein, 10 aa, Merkel Cell Polyoma Virus
  PEPTIDE (1)..(10): VP1
TVYPKPSVAP

SEQ ID NO: 159 - protein, 9 aa, Merkel Cell Polyoma Virus
  PEPTIDE (1)..(9): VP1
GVEVLSVVT

SEQ ID NO: 160 - protein, 9 aa, Merkel Cell Polyoma Virus
  PEPTIDE (1)..(9): VP1
PLDLQGLVL

SEQ ID NO: 161 - protein, 9 aa, Merkel Cell Polyoma Virus
  PEPTIDE (1)..(9): VP1
GLDPQAKAK

SEQ ID NO: 162 - protein, 9 aa, Merkel Cell Polyoma Virus
  PEPTIDE (1)..(9): VP1
EVWCPDPSK

SEQ ID NO: 163 - protein, 9 aa, Merkel Cell Polyoma Virus
  PEPTIDE (1)..(9): VP1
ADIVGFLFK

SEQ ID NO: 164 - protein, 9 aa, Merkel Cell Polyoma Virus
  PEPTIDE (1)..(9): VP1
KTSGKMALH

SEQ ID NO: 165 - protein, 9 aa, Merkel Cell Polyoma Virus
  PEPTIDE (1)..(9): VP1
KMALHGLPR

SEQ ID NO: 166 - protein, 9 aa, Merkel Cell Polyoma Virus
  PEPTIDE (1)..(9): VP1
RYFNVTLRK

SEQ ID NO: 167 - protein, 9 aa, Merkel Cell Polyoma Virus
  PEPTIDE (1)..(9): VP1
TLRKRWVKN

SEQ ID NO: 168 - protein, 10 aa, Human cytomegalovirus
  PEPTIDE (1)..(10): CMV  pp65  RPH-L
RPHERNGFTV

SEQ ID NO: 169 - protein, 9 aa, Human herpesvirus 4
  PEPTIDE (1)..(9): EBV  EBNA  RPP
RPPIFIRLL

SEQ ID NO: 170 - protein, 9 aa, Merkel Cell Polyoma Virus
  PEPTIDE (1)..(9): VP1
KPGCCPNVA

SEQ ID NO: 171 - protein, 9 aa, Merkel Cell Polyoma Virus
  PEPTIDE (1)..(9): VP1
QPIKENLPA

SEQ ID NO: 172 - protein, 9 aa, Merkel Cell Polyoma Virus
  PEPTIDE (1)..(9): VP1
LPRYFNVTL

SEQ ID NO: 173 - protein, 9 aa, Merkel Cell Polyoma Virus
  PEPTIDE (1)..(9): VP1
MPKVSGQPM

SEQ ID NO: 174 - protein, 9 aa, Merkel Cell Polyoma Virus
  PEPTIDE (1)..(9): VP1
YPKPSVAPA

SEQ ID NO: 175 - protein, 9 aa, Merkel Cell Polyoma Virus
  PEPTIDE (1)..(9): VP1
KPSVAPAAV

SEQ ID NO: 176 - protein, 9 aa, Merkel Cell Polyoma Virus
  PEPTIDE (1)..(9): VP1
APLKGPQKA

SEQ ID NO: 177 - protein, 10 aa, Merkel Cell Polyoma Virus
  PEPTIDE (1)..(10): VP1
APKRKASSTC

SEQ ID NO: 178 - protein, 10 aa, Merkel Cell Polyoma Virus
  PEPTIDE (1)..(10): VP1
SVARVSLPML

SEQ ID NO: 179 - protein, 10 aa, Merkel Cell Polyoma Virus
  PEPTIDE (1)..(10): VP1
YPKTTNGGPI

SEQ ID NO: 180 - protein, 10 aa, Merkel Cell Polyoma Virus
  PEPTIDE (1)..(10): VP1
YPKPSVAPAA

SEQ ID NO: 181 - protein, 11 aa, Merkel Cell Polyoma Virus
  PEPTIDE (1)..(11): VP1
KPGCCPNVASV

SEQ ID NO: 182 - protein, 11 aa, Merkel Cell Polyoma Virus
  PEPTIDE (1)..(11): VP1
NPRMGVNSPDL

SEQ ID NO: 183 - protein, 11 aa, Merkel Cell Polyoma Virus
  PEPTIDE (1)..(11): VP1
LPAYSVARVSL

SEQ ID NO: 184 - protein, 11 aa, Merkel Cell Polyoma Virus
  PEPTIDE (1)..(11): VP1
TPTVLQFSNTL

SEQ ID NO: 185 - protein, 11 aa, Merkel Cell Polyoma Virus
  PEPTIDE (1)..(11): VP1
LPRYFNVTLRK

SEQ ID NO: 186 - protein, 11 aa, Merkel Cell Polyoma Virus
  PEPTIDE (1)..(11): VP1
YPVVNLINSLF

SEQ ID NO: 187 - protein, 11 aa, Merkel Cell Polyoma Virus
  PEPTIDE (1)..(11): VP1
YPKPSVAPAAV

SEQ ID NO: 188 - protein, 11 aa, Merkel Cell Polyoma Virus
  PEPTIDE (1)..(11): VP1
KPSVAPAAVTF

SEQ ID NO: 189 - protein, 9 aa, Merkel Cell Polyoma Virus
  PEPTIDE (1)..(9): VP1
APKRKASST